European Patent Application EP 4 597 114 A1, published August 6, 2025. Title: Methods for in vitro prognosis, diagnosis and evaluation of muscle dysfunction and/or prognosis of muscle efficiency in a subject. Applicant: Université Paris Cité. The sequence listing filed with the application follows.

SEQUENCE LISTING (3 sequences)

SEQ ID NO: 1 - DNA, 20 bp, synthetic construct
  source 1..20: mol_type = other DNA
ggcttctggtcaagggacaa

SEQ ID NO: 2 - DNA, 21 bp, synthetic construct
  source 1..21: mol_type = other DNA
tgcttgcatgtaggccagata

SEQ ID NO: 3 - DNA, 7973 bp, synthetic construct
  source 1..7973: mol_type = other DNA
atatagcataaatcaatattggctattggccattgcatacgttgtatccatatcataatatgtacatttatattggctcatgtccaacattaccgccatgttgacattgattattgactagttattaatagtaatcaattacggggtcattagttcatagcccatatatggagttccgcgttacataacttacggtaaatggcccgcctggctgaccgcccaacgacccccgcccattgacgtcaataatgacgtatgttcccatagtaacgccaatagggactttccattgacgtcaatgggtggagtatttacggtaaactgcccacttggcagtacatcaagtgtatcatatgccaagtacgccccctattgacgtcaatgacggtaaatggcccgcctggcattatgcccagtacatgaccttatgggactttcctacttggcagtacatctacgtattagtcatcgctattaccatggtgatgcggttttggcagtacatcaatgggcgtggatagcggtttgactcacggggatttccaagtctccaccccattgacgtcaatgggagtttgttttggcaccaaaatcaacgggactttccaaaatgtcgtaacaactccgccccattgacgcaaatgggcggtaggcgtgtacggtgggaggtctatataagcagagctcgtttagtgaaccgtcagatcgcctggagacgccatccacgctgttttgacctccatagaagacaccgggaccgatccagcctccgcggccccaagcttgaattctctactttgcccgcccacagatgtagttttctctgcgcgtgtgcgttttccctcctccccgccctcagggtccacggccaccatggcgtattaggggcagcagtgcctgcggcagcattggcctttgcagcggcggcagcagcaccaggctctgcagcggcaacccccagcggcttaagccatggcgcttctcacggcattcagcagcagcgttgctgtaaccgacaaagacaccttcgaattaagcacattcctcgattccagcaaagcaccgcaacatgaccgaaatgagcttcctgagcagcgaggtgttggtgggggacttgatgtcccccttcgaccagtcgggtttgggggctgaatacccctacgacgtgcccgactacgccggtggatcagggggaggatccgtctccaaaggggaagcggtcattaaagagttcatgaggttcaaagttcatatggagggcagtatgaacggccatgaatttgaaatcgagggcgagggggagggacgcccttacgaagggacacaaacagccaaactgaaggttacgaaaggtgggccacttccctttagttgggatatactgtcacctcaatttatgtacggcagccgagccttcattaaacatcccgctgacattccggattactataagcagtcctttccagaggggtttaaatgggagcgggttatgaatttcgaggatggcggggccgtaactgtcacgcaggataccagtctggaagatggtaccctgatttataaggttaagctcagaggaacgaacttcccgccagatggtcccgtaatgcaaaaaaagacgatgggttgggaggcatcaactgaaagattgtatcctgaggatggtgtccttaagggtgatattaaaatggctctgaggctgaaggatggcggaaggtatttggcagatttcaaaactacatataaggccaagaagcctgttcagatgccaggtgcctataatgtggacagaaaacttgacattacatcacacaacgaggattataccgtcgtggagcaatatgagagaagtgagggccgacatagtaccggcggcatggatgaactctataaggtcgacggtggatcagggggacccgccgccaagcgcgtgaagctggactaatctagaatcgataaaataaaagattttatttagtctccagaaaaaggggggaatgaaagaccccacctgtaggtttggcaagctagcttaagtaacgccattttgcaaggcatggaaaaatacataactgagaatagagaagttcagatcaaggtcaggaacagatggaacagctgaatatgggccaaacaggatatctgtggtaagcagttcctgccccggctcagggccaagaacagatggaacagctgaatatgggccaaacaggatatctgtggtaagcagttcctgccccggctcagggccaagaacagatggtccccagatgcggtccagccctcagcagtttctagagaaccatcagatgtttccagggtgccccaaggacctgaaatgaccctgtgccttatttgaactaaccaatcagttcgcttctcgcttctgttcgcgcgcttctgctccccgagctcaataaaagagcccacaacccctcactcggggcgccagtcctccgattgactgagtcgcccgggtacccgtgtatccaataaaccctcttgcagttgcatccgacttgtggtctcgctgttccttgggagggtctcctctgagtgattgactacccgtcagcgggggtctttcatttgggggctcgtccgggatcgggagacccctgcccagggaccaccgacccaccaccgggaggtaagctggctgcctcgcgcgtttcggtgatgacggtgaaaacctctgacacatgcagctcccggagacggtcacagcttgtctgtaagcggatgccgggagcagacaagcccgtcagggcgcgtcagcgggtgttggcgggtgtcggggcgcagccatgacccagtcacgtagcgatagcggagtgtatactggcttaactatgcggcatcagagcagattgtactgagagtgcaccatatgcggtgtgaaataccgcacagatgcgtaaggagaaaataccgcatcaggcgctcttccgcttcctcgctcactgactcgctgcgctcggtcgttcggctgcggcgagcggtatcagctcactcaaaggcggtaatacggttatccacagaatcaggggataacgcaggaaagaacatgtgagcaaaaggccagcaaaaggccaggaaccgtaaaaaggccgcgttgctggcgtttttccataggctccgcccccctgacgagcatcacaaaaatcgacgctcaagtcagaggtggcgaaacccgacaggactataaagataccaggcgtttccccctggaagctccctcgtgcgctctcctgttccgaccctgccgcttaccggatacctgtccgcctttctcccttcgggaagcgtggcgctttctcatagctcacgctgtaggtatctcagttcggtgtaggtcgttcgctccaagctgggctgtgtgcacgaaccccccgttcagcccgaccgctgcgccttatccggtaactatcgtcttgagtccaacccggtaagacacgacttatcgccactggcagcagccactggtaacaggattagcagagcgaggtatgtaggcggtgctacagagttcttgaagtggtggcctaactacggctacactagaaggacagtatttggtatctgcgctctgctgaagccagttaccttcggaaaaagagttggtagctcttgatccggcaaacaaaccaccgctggtagcggtggtttttttgtttgcaagcagcagattacgcgcagaaaaaaaggatctcaagaagatcctttgatcttttctacggggtctgacgctcagtggaacgaaaactcacgttaagggattttggtcatgagattatcaaaaaggatcttcacctagatccttttaaattaaaaatgaagttttaaatcaatctaaagtatatatgagtaaacttggtctgacagttaccaatgcttaatcagtgaggcacctatctcagcgatctgtctatttcgttcatccatagttgcctgactccccgtcgtgtagataactacgatacgggagggcttaccatctggccccagtgctgcaatgataccgcgagacccacgctcaccggctccagatttatcagcaataaaccagccagccggaagggccgagcgcagaagtggtcctgcaactttatccgcctccatccagtctattaattgttgccgggaagctagagtaagtagttcgccagttaatagtttgcgcaacgttgttgccattgctgcaggcatcgtggtgtcacgctcgtcgtttggtatggcttcattcagctccggttcccaacgatcaaggcgagttacatgatcccccatgttgtgcaaaaaagcggttagctccttcggtcctccgatcgttgtcagaagtaagttggccgcagtgttatcactcatggttatggcagcactgcataattctcttactgtcatgccatccgtaagatgcttttctgtgactggtgagtactcaaccaagtcattctgagaatagtgtatgcggcgaccgagttgctcttgcccggcgtcaacacgggataataccgcgccacatagcagaactttaaaagtgctcatcattggaaaacgttcttcggggcgaaaactctcaaggatcttaccgctgttgagatccagttcgatgtaacccactcgtgcacccaactgatcttcagcatcttttactttcaccagcgtttctgggtgagcaaaaacaggaaggcaaaatgccgcaaaaaagggaataagggcgacacggaaatgttgaatactcatactcttcctttttcaatattattgaagcatttatcagggttattgtctcatgagcggatacatatttgaatgtatttagaaaaataaacaaataggggttccgcgcacatttccccgaaaagtgccacctgacgtctaagaaaccattattatcatgacattaacctataaaaataggcgtatcacgaggccctttcgtcttcaagaattcataccagatcaccgaaaactgtcctccaaatgtgtccccctcacactcccaaattcgcgggcttctgcctcttagaccactctaccctattccccacactcaccggagccaaagccgcggcccttccgtttctttgcttttgaaagaccccacccgtaggtggcaagctagcttaagtaacgccactttgcaaggcatggaaaaatacataactgagaatagaaaagttcagatcaaggtcaggaacaaagaaacagctgaataccaaacaggatatctgtggtaagcggttcctgccccggctcagggccaagaacagatgagacagctgagtgatgggccaaacaggatatctgtggtaagcagttcctgccccggctcggggccaagaacagatggtccccagatgcggtccagccctcagcagtttctagtgaatcatcagatgtttccagggtgccccaaggacctgaaaatgaccctgtaccttatttgaactaaccaatcagttcgcttctcgcttctgttcgcgcgcttccgctctccgagctcaataaaagagcccacaacccctcactcggcgcgccagtcttccgatagactgcgtcgcccgggtacccgtattcccaataaagcctcttgctgtttgcatccgaatcgtggtctcgctgttccttgggagggtctcctctgagtgattgactacccacgacgggggtctttcatttgggggctcgtccgggatttggagacccctgcccagggaccaccgacccaccaccgggaggtaagctggccagcaacttatctgtgtctgtccgattgtctagtgtctatgtttgatgttatgcgcctgcgtctgtactagttagctaactagctctgtatctggcggacccgtggtggaactgacgagttctgaacacccggccgcaaccctgggagacgtcccagggactttgggggccgtttttgtggcccgacctgaggaagggagtcgatgtggaatccgaccccgtcaggatatgtggttctggtaggagacgagaacctaaaacagttcccgcctccgtctgaatttttgctttcggtttggaaccgaagccgcgcgtcttgtctgctgcagcgctgcagcatcgttctgtgttgtctctgtctgactgtgtttctgtatttgtctgaaaattagggccagactgttaccactcccttaagtttgaccttaggtcactggaaagatgtcgagcggatcgctcacaaccagtcggtagatgtcaagaagagacgttgggttaccttctgctctgcagaatggccaacctttaacgtcggatggccgcgagacggcacctttaaccgagacctcatcacccaggttaagatcaaggtcttttcacctggcccgcatggacacccagaccaggtcccctacatcgtgacctgggaagccttggcttttgacccccctccctgggtcaagccctttgtacaccctaagcctccgcctcctcttcctccatccgccccgtctctcccccttgaacctcctcgttcgaccccgcctcgatcctccctttatccagccctcactccttctctaggcgccggaattccgatctgatagcttgccacaacccgtaccaaagatggatagatccggaaagcctgaactcaccgcgacgtctgtcgagaagtttctgatcgaaaagttcgacagcgtctccgacctgatgcagctctcggagggcgaagaatctcgtgctttcagcttcgatgtaggagggcgtggatatgtcctgcgggtaaatagctgcgccgatggtttctacaaagatcgttatgtttatcggcactttgcatcggccgcgctcccgattccggaagtgcttgacattggggaattcagcgagagcctgacctattgcatctcccgccgtgcacagggtgtcacgttgcaagacctgcctgaaaccgaactgcccgctgttctgcagccggtcgcggaggccatggatgcgatcgctgcggccgatcttagccagacgagcgggttcggcccattcggaccgcaaggaatcggtcaatacactacatggcgtgatttcatatgcgcgattgctgatccccatgtgtatcactggcaaactgtgatggacgacaccgtcagtgcgtccgtcgcgcaggctctcgatgagctgatgctttgggccgaggactgccccgaagtccggcacctcgtgcacgcggatttcggctccaacaatgtcctgacggacaatggccgcataacagcggtcattgactggagcgaggcgatgttcggggattcccaatacgaggtcgccaacatcttcttctggaggccgtggttggcttgtatggagcagcagacgcgctacttcgagcggaggcatccggagcttgcaggatcgccgcggctccgggcgtatatgctccgcattggtcttgaccaactctatcagagcttggttgacggcaatttcgatgatgcagcttgggcgcagggtcgatgcgacgcaatcgtccgatccggagccgggactgtcgggcgtacacaaatcgcccgcagaagcgcggccgtctggaccgatggctgtgtagaagtactcgccgatagtggaaaccgacgccccagcactcgtccgagggcaaaggaatagagtagatgccgaccgaacaagagctgatttcgagaacgcctcagccagcaactcgcgcgagcctagcaaggcaaatgcgagagaacggccttacgcttggtggcacagttctcgtccacagttcgctaagctcgctcggctgggtcgcgggagggccggtcgcagtgattcaggcccttctggattgtgttggtccccagggcacgattgtcatgcccacgcactcgggtgatctgactgatcccgcagattggagatcgccgcccgtgcctgccgattgggtgcagatctctagagctcgctgatccggccattagccatattattcattggtt